European Patent Application EP 4 578 944 A1, published July 2, 2025. Title: Aminoacyl tRNA synthetase mutant and use thereof. Applicant: Asymchem Laboratories (Tianjin) Co., Ltd. Application CN. The sequence listing filed with the application follows.

SEQUENCE LISTING (19 sequences)

SEQ ID NO: 1 - DNA, 561 bp, synthetic construct
  source 1..561: mol_type = other DNA; note = mcherry sequnce
ccatgggcatggttagcaaaggcgaagaagataacatggccatcatcaaggagttcatgcgcttcaaggtgcacatggagggcagcgtgaacggccatgagtttgaaatcgagggcgaaggcgaaggtcgcccatacgaaggcacccagaccgccaaactgaaagtgacgaaaggcggtccgctgccattcgcgtgggatattctgagcccacagttcatgtacggcagcaaagcctacgtgaagcatccggccgatatcccggattatctgaagctgagcttcccagagggcttcaagtgggagcgcgtgatgaactttgaagatggcggtgtggttaccgttacgcaagatagcagtctgcaagatggcgagttcatctacaaggttaagctccgcggcaccaacttcccgagcgatggtccggtgatgcagaaaaagacgatgggctgggaagcgagcagcgaacgcatgtatccagaagatggcgcgctgaaaggcgagatcaaacagcgtctgaagctgaaagacggcggccattacgatgcggaggtgactcgag

SEQ ID NO: 2 - DNA, 47 bp, synthetic construct
  source 1..47: mol_type = other DNA; note = primer
gagtcgtattaatttcgcgggatcgagtgagcgcaacgcaattaatg

SEQ ID NO: 3 - DNA, 42 bp, synthetic construct
  source 1..42: mol_type = other DNA; note = primer
gcattaagcgcggcgggtgtggtgttttcaccgtcatcaccg

SEQ ID NO: 4 - DNA, 47 bp, synthetic construct
  source 1..47: mol_type = other DNA; note = primer
cattaattgcgttgcgctcactcgatcccgcgaaattaatacgactc

SEQ ID NO: 5 - DNA, 42 bp, synthetic construct
  source 1..42: mol_type = other DNA; note = primer
cggtgatgacggtgaaaacaccacacccgccgcgcttaatgc

SEQ ID NO: 6 - DNA, 444 bp, synthetic construct
  source 1..444: mol_type = other DNA; note = a promoter and a terminator
agatctgagctcccggtcatcaatcatccccataatccttgttagatgatcaattttaaaaaactaacagttcagcctgtcccgcttataagatccgttatacgtttacgctttgaggaatcccatcatatggaattcctgcagtttcaaacgctaaattgcctgatgcgctacgcttatcaggcctacatgatctctgatatattgagtacgtcttttgtaggccggataatcgttcactcgcatccggcagaaacagcaacatccaaaacgccgcgttcagcggcgtttatgcttttcttcgcgaattaattccgcttcgcaacatgtgagcaccggtttattgactaccggaagcagtgtgaccgtgtgctttaaatgcctgaggccagtttgctcaggctctccccgtggaggtaataattgacgatatgatcactcgag

SEQ ID NO: 7 - DNA, 921 bp, synthetic construct
  source 1..921: mol_type = other DNA; note = MjTyrRS sequence
atggatgaatttgaaatgattaaacgcaacaccagcgaaattattagcgaagaagaactgcgcgaagtgctgaagaaggacgagaagtcagcttatattggctttgaaccgagcggcaagatacacctgggccattatttacagattaagaagatgatcgatttacagaacgcgggctttgatattattattctgctggcggatctgcatgcgtatctgaaccagaaaggcgaactggatgaaattcgcaagatcggagattataacaagaaggtatttgaggcgatgggcctgaaagcgaaatatgtgtatggcagcgagtttcagctggataaagattataccctgaacgtgtatcgcctggcgctgaagacgacactgaaacgcgcgcgccgcagcatggaactgattgcgcgcgaagatgagaatcccaaagtggcggaagtgatttatccgattatgcaggtgaacgatattcactatctgggcgtggatgtggcggtgggcggcatggaacagcgcaagatacacatgctggcgcgcgaactgctgccgaagaaggtagtttgcattcataacccggtgctgaccggcctggatggcgaaggcaagatgtccagcagcaaaggcaactttattgcggtggatgatagcccggaagaaattcgcgcgaagatcaagaaagcgtactgcccggcgggcgtggtggaaggcaacccgattatggaaattgcgaaatatttcttagagtatccgctgaccattaaacgcccggagaagttcggtggcgatctgaccgtgaacagctatgaagaactggaaagcctgtttaagaataaggaactgcatccgatggatctgaagaatgctgtggcggaagaactgattaagatactcgaaccgattcgcaaacgcctgtaa

SEQ ID NO: 8 - DNA, 56 bp, synthetic construct
  source 1..56: mol_type = other DNA; note = primer
gctgaagaaggacgagaagtcannknnkattggctttgaaccgagcggcaagatac

SEQ ID NO: 9 - DNA, 61 bp, synthetic construct
  source 1..61: mol_type = other DNA; note = primer
tctggttcagatacgcatgmnnatcmnncagmnnaataataatatcaaagcccgcgttctg

SEQ ID NO: 10 - DNA, 64 bp, synthetic construct
  source 1..64: mol_type = other DNA; note = primer
gggctttgatattattattnnkctgnnkgatnnkcatgcgtatctgaaccagaaaggcgaactg

SEQ ID NO: 11 - DNA, 70 bp, synthetic construct
  source 1..70: mol_type = other DNA; note = primer
cacgttcagggtataatctttatcmnnmnnmnnmnngctgccatacacatatttcgctttcaggcccatc

SEQ ID NO: 12 - DNA, 66 bp, synthetic construct
  source 1..66: mol_type = other DNA; note = primer
gcgaaatatgtgtatggcagcnnknnknnknnkgataaagattataccctgaacgtgtatcgcctg

SEQ ID NO: 13 - DNA, 75 bp, synthetic construct
  source 1..75: mol_type = other DNA; note = primer
catgccgcccaccgccacatccacgccmnnmnnmnnmnnmnngttcacctgcataatcggataaatcacttccgc

SEQ ID NO: 14 - DNA, 28 bp, synthetic construct
  source 1..28: mol_type = other DNA; note = primer
tgacttctcgtccttcttcagcacttcg

SEQ ID NO: 15 - DNA, 22 bp, synthetic construct
  source 1..22: mol_type = other DNA; note = primer
ggatgtggcggtgggcggcatg

SEQ ID NO: 16 - DNA, 720 bp, synthetic construct
  source 1..720: mol_type = other DNA; note = sfGFP gene sequence
atgagcaaaggtgaagaactgtttaccggcgttgtgccgattctggtggaactggatggcgatgtgaacggtcacaaattcagcgtgcgtggtgaaggtgaaggcgatgccacgattggcaaactgacgctgaaatttatctgcaccaccggcaaactgccggtgccgtggccgacgctggtgaccaccctgacctatggcgttcagtgttttagtcgctatccggatcacatgaaacgtcacgatttctttaaatctgcaatgccggaaggctatgtgcaggaacgtacgattagctttaaagatgatggcaaatataaaacgcgcgccgttgtgaaatttgaaggcgataccctggtgaaccgcattgaactgaaaggcacggattttaaagaagatggcaatatcctgggccataaactggaatacaactttaatagccataatgtttatattacggcggataaacagaaaaatggcatcaaagcgaattttaccgttcgccataacgttgaagatggcagtgtgcagctggcagatcattatcagcagaataccccgattggtgatggtccggtgctgctgccggataatcattatctgagcacgcagaccgttctgtctaaagatccgaacgaaaaaggcacgcgggaccacatggttctgcacgaatatgtgaatgcggcaggtattacgtggagccatccgcagttcgaaaaa

SEQ ID NO: 17 - DNA, 32 bp, synthetic construct
  source 1..32: mol_type = other DNA; note = primer
gggctcgagcccatcaaaaaaatattctcaac

SEQ ID NO: 18 - DNA, 31 bp, synthetic construct
  source 1..31: mol_type = other DNA; note = primer
gggctcgagtaaaaaaaatccttagctttcg

SEQ ID NO: 19 - protein, 306 aa, synthetic construct
  source 1..306: note = a MjTyrRS-encoded protein
MDEFEMIKRNTSEIISEEELREVLKKDEKSAYIGFEPSGKIHLGHYLQIKKMIDLQNAGFDIIILLADLHAYLNQKGELDEIRKIGDYNKKVFEAMGLKAKYVYGSEFQLDKDYTLNVYRLALKTTLKRARRSMELIAREDENPKVAEVIYPIMQVNDIHYLGVDVAVGGMEQRKIHMLARELLPKKVVCIHNPVLTGLDGEGKMSSSKGNFIAVDDSPEEIRAKIKKAYCPAGVVEGNPIMEIAKYFLEYPLTIKRPEKFGGDLTVNSYEELESLFKNKELHPMDLKNAVAEELIKILEPIRKRL